European Patent Specification EP 3 223 846 B1, published September 6, 2023. Title: ADJUADJUVANT COMPOSITIONS AND RELATED METHODS. Applicant: VaxLiant, LLC Miller, Timothy J Pfannenstiel, Mary Ann. The sequence listing filed with the application follows.

SEQUENCE LISTING (1 sequence)

SEQ ID NO: 1 - protein, 12 aa, Avian influenza virus
  MISC_FEATURE: Sequence is a HP multibasic cleavage site
PLRERRRKRGLF